European Patent Specification EP 3 948 285 B1, published September 3, 2025. Title: SALIVARY BIOMARKERS FOR THE DETECTION OF HEAD AND NECK EPIDERMOID CANCER (CECC). Applicant: Bioithas S.L. The sequence listing filed with the application follows.

SEQUENCE LISTING (21 sequences)

SEQ ID NO: 1 - DNA, 418 bp, Alloprevotella
  misc_feature (1)..(418): Representative sequence.
aggaatattggtcaatggacggaagtctgaaccagccaagtagcgtgcaggatgacggccctctgggttgtaaactgcttttagttgggaataaaaaagaggacgtgtcctctattgtatgtaccttcagaaaaaggaccggctaattccgtgccagcagccgcggtaatacggaaggtccaggcgttatccggatttattgggtttaaagggagcgtaggcggattattaagtcagtggtgaaagacggtggctcaaccatcgttagccattgaaactggtagtcttgagtgcagacagggatgctggaactcgtggtgtagcggtgaaatgcttagatatgacgaagaactccgattgcgaaggcagctgacgggagcgcaactgacgcttaagctcgaaggtgcgggtatcaaac

SEQ ID NO: 2 - DNA, 418 bp, Alloprevotella
  misc_feature (1)..(418): Representative sequence
aggaatattggtcaatggacggaagtctgaaccagccaagtagcgtgcaggatgacggccctctgggttgtaaactgcttttagttgggaataaaaaagaggacgtgtcctctattgtatgtaccttcagaaaaaggaccggctaattccgtgccagcagccgcggtaatacggaaggtccaggcgttatccggatttattgggtttaaagggagcgtaggcggattattaagtcagtggtgaaagacggtggctcaaccatcgttagccattgaaactggtagtcttgagtgcagacagggatgctggaactcgtggtgtagcggtgaaatgcttagatatcacgatgaactccaatcgcgaaggcaggtgtccgggctgcaactgacgctgaggctcgaaagtgtgggtatcaaac

SEQ ID NO: 3 - DNA, 418 bp, Alloprevotella
  misc_feature (1)..(418): Representative sequence
aggaatattggtcaatggacggaagtctgaaccagccaagtagcgtgcaggatgacggccctctgggttgtaaactgcttttagttgggaataaaaaagaggacgtgtcctctattgtatgtaccttcagaaaaaggaccggctaattccgtgccagcagccgcggtaatacggaaggtccaggcgttatccggatttattgggtttaaagggagcgtaggcggattattaagtcagtggtgaaagacggtggctcaaccatcgttagccattgaaactggtagtcttgagtgcagacagggatgctggaactcgtggtgtagcggtgaaatgcttagatatcacgatgaactccgatcgcgaaggcaggtgtccgggctgcaactgacgctgaggctcgaaagtgtgggtatcaaac

SEQ ID NO: 4 - DNA, 400 bp, Prevotella
  misc_feature (1)..(400): Representative sequence
gggaatattgcacaatgggggaaaccctgatgcagcaacgccgcgtgaacgatgaaggcctttgggtcgtaaagttctgttctaggtgatgaaaactgacagtaacctaggagaaagccccggctaactccgtgccagcagccgcggtaatacggagggggcaagcgttatccggatttattgggtttaaagggagcgtaggccgtagattaagcgtgttgtgaaatgtagatgctcaacatctgacttgcagcgcgaactggtttacttgagtgtgcgcaacgtaggcggaattcgtcgtgtagcggtgaaatgcttagatatgacgaagaactccgattgcgaaggcagcttacgggagcacaactgacgctgaagctcgaaggtgcgggtatcaaac

SEQ ID NO: 5 - DNA, 397 bp, Prevotella
  misc_feature (1)..(397): Representative sequence.
gggaatattgcacaatggaggaaactctgatgcagtgacaccgcgtataggaagaaggtcttaggattgtaagctattgtcgtgtgagaagaaaatgaccatcacaggaggaagccctggctaaatatgtgccagcagccgcggtaatacggaaggtccgggcgttatccggatttattgggtttaaagggagcgtaggccgtggattaagcgtgttgtgaaatgcaggtgctcaacgtctgcactgcagcgcgaactggttcacttgagtgtgcacaacgcaggcggaattcgtcgtgtagcggtgaaatgcttagatatgacgaagaactccgattgcgaaggcagcttgcgggagcacaactgacgctgaagctcgaaagtgcgggtatcgaac

SEQ ID NO: 6 - DNA, 402 bp, Prevotella
  misc_feature (1)..(402): Representative sequence
gggaatattggacaatgggggcaaccctgatccagcaattctgtgtgcacgatgaaggtcttcggattgtaaagtgctttcagcagggaagaaaaaaatgacggtacctgcagaagaagcgacggctaaatacgtgccagcagccgcggtaatacggaaggtccaggcgttatccggatttattgggtttaaagggagtgtaggcggtttgttaagcgtgttgtgaaatttagatgctcaacatttaacttgcagcgcgaactgtcagacttgagtacacgcaacgtatgcggaattcatggtgtagcggtgaaatgcttagatatcatgaagaactccgattgcgaaggcagcatacgggagtgtaactgacgcttaagctcgaaggtgcgggtatcgaac

SEQ ID NO: 7 - DNA, 400 bp, Campylobacter
  misc_feature (1)..(400): Representative sequence
gggaatattgctcaatgggggaaaccctgaagcagcaacgccgcgtggaggatgacacttttcggagcgtaaactccttttcttggggaagaaatttgacggtacccaaggaataagcaccggctaactccgtgccagcagccgcggtaatacggagggtgcaagcgttactcggaatcactgggcgtaaaggacgcgtaggcggattatcaagtctcttgtgaaatccaatggcttaaccattgaactgcttgggaaactgataatctagagtgagggagaggcagatggaattggtggtgtaggggtaaaatccgtagagatcaccaggaatacccattgcgaaggcgatctgctggaactcaactgacgctaatgcgtgaaagcgtggggagcaaac

SEQ ID NO: 8 - DNA, 400 bp, Campylobacter
  misc_feature (1)..(400): Representative sequence
gggaatattgctcaatgggggaaaccctgaagcagcaacgccgcgtggaggatgacacttttcggagcgtaaactccttttcttggggaagaaatttgacggtacccaaggaataagcaccggctaactccgtgccagcagccgcggtaatacggagggtgcaagcgttactcggaatcactgggcgtaaaggacgcgtaggcggattatcaagtctcttgtgaaatccaatggcttaaccattgaactgcttgggaaactgataatctagagtgagggagaggcagatggaattggtggtgtaggggtaaaatccgtagagatcaccaggaatacccattgcgaaggcgatctgctggaactcaactgacgctaatgcgcgaaagcgtggggagcaaac

SEQ ID NO: 9 - DNA, 400 bp, Campylobacter
  misc_feature (1)..(400): Representative sequence
gggaatattgctcaatgggggaaaccctgaagcagcaacgccgcgtggaggatgacacttttcggagcgtaaactccttttcttaggaaagaattatgacggtacctaaggaataagcaccggctaactccgtgccagcagccgcggtaatacggggggtgcaagcgttactcggaatcactgggcgtaaaggacgcgtaggcggattatcaagtctcttgtgaaatttaacggcttaaccgttaaactgcttgggaaactgataatctagagtaagggagaggcagatggaattcttggtgtaggggtaaaatccgtagagatcaagaagaatacttattgcgaaggcgatctgctagaacttaactgacgctaatgcgtgaaagcgtggggagcaaac

SEQ ID NO: 10 - DNA, 405 bp, Rothia
  misc_feature (1)..(405): Representative sequence
gggaatcttcggcaatggacggaagtctgaccgagcaacgccgcgtgagtgaagaaggttttcggatcgtaaagctctgttagcagggaagaagagagattgacggtacctgcagagaaagcgccggctaactacgtgccagcagccgcggtaatacgtagggcgcgagcgttgtccggaattattgggcgtaaagagcttgtaggcggtttgtcgcgtctgctgtgaaaggccggagcttaactccgtgtattgcagtgggtacgggcagactagagtgcagtaggggagactggaactcctggtgtagcggtggaatgcgcagatatcaggaagaacaccgatggcgaaggcaggtctctgggctgtaactgacgctgagaagcgaaagcatggggagcgaac

SEQ ID NO: 11 - DNA, 406 bp, Rothia
  misc_feature (1)..(406): Representative sequence
aggaatattggtcaatgggcgcgagcctgaaccagccaagtagcgtgcaggatgacggccctatgggttgtaaacctctgttagcagggaagaagagagattgacggtacctgcagagaaagcgccggctaactacgtgccagcagccgcggtaatacgtagggcgcgagcgttgtccggaattattgggcgtaaagagcttgtaggcggtttgtcgcgtctgctgtgaaaggccggagcttaactccgtgtattgcagtgggtacgggcagactagagtgcagtaggggagactggaattcctggtgtagcggtggaatgcgcagatatcaggaggaacaccgatggcgaaggcaggtctctgggctgtaactgacgctgagaagcgaaagcatggggagcgaac

SEQ ID NO: 12 - DNA, 405 bp, Rothia
  misc_feature (1)..(405): Representative sequence
gggaatattgcacaatgggcgcaagcctgatgcagcgacgccgcgtgagggatgacggccttcgggttgtaaacctctgttagcagggaagaagagagattgacggtacctgcagagaaagcgccggctaactacgtgccagcagccgcggtaatacgtagggcgcgagcgttgtccggaattattgggcgtaaagagcttgtaggcggtttgtcgcgtctgctgtgaaaggccggagcttaactccgtgtattgcagtgggtacgggcagactagagtgcagtaggggagactggaattcctggtgtagcggtgaaatgcgtagatattaggaagaacaccagtggcgaaggcgactttctggacgaaaactgacgctgaggcgcgaaagccaggggagcgaac

SEQ ID NO: 13 - DNA, 399 bp, Catonella
  misc_feature (1)..(399): Representative sequence
ggggatattgcacaatggaggaaactctgatgcagcgacgccgcgtgagtgaagaagtgctccggcatgtaaagctctttcagcagggaagatgatgacggtacctgaataagaagccccggctaactacgtgccagcagccgcggtaatacgtagggggcaagcgttatccggatttactgggtgtaaagggagcgcaggcggtctggcaagttgagagtggaagcagggggctcaaccccctgactgctcccaaaactgttggactggagtatgggagaggcaggcggaattcctagtgtagcggtgaaatgctcagatattaggaagaacaccggtggcgaaggcggcctgctggaccaaaactgacgctgaggctcgagagcgtggggagcgaac

SEQ ID NO: 14 - DNA, 399 bp, Catonella
  misc_feature (1)..(399): Representative sequence
ggggatattgcacaatggaggaaactctgatgcagcgacgccgcgtgagtgaagaagtatttcggtatgtaaagctctatcagcagggaagatgatgacggtacctgactaagaagccccggctaactacgtgccagcagccgcggtaatacgtagggggcaagcgttatccggatttactgggtgtaaagggagcgcaggcggttttgcaagttgagagtggaagcagggggctcaaccccttgactgctcccaaaactgtaaaacttgagtgtagatgaggtaggcggaatgcgtggtgtagcggtggaatgcatagatatcacgcagaactccgattgcgaaggcagcttactaaggtacaactgacgctgaagcacgaaagcgtgggtatcaaac

SEQ ID NO: 15 - DNA, 399 bp, Catonella
  misc_feature (1)..(399): Representative sequence
ggggatattgcacaatggaggaaactctgatgcagcgacgccgcgtgagtgaagaagtatttcggtatgtaaagctctatcagcagggaagatgatgacggtacctgactaagaagccccggctaactacgtgccagcagccgcggtaatacgtagggggcaagcgttatccggatttactgggtgtaaagggagcgcaggcggttttgcaagttgagagtggaagcagggggctcaaccccctgactgctcccaaaactgtaaaacttgagtatgggagaggcaggcggaattcctagtgtagcggtgaaatgcttagatattaggaagaacaccggtggcgaaggcggcctgctggaccaaaactgacgctgaggctcgaaagcgtgggtagcaaac

SEQ ID NO: 16 - DNA, 418 bp, Porphyromona
  misc_feature (1)..(418): Representative sequence
aggaatattggtcaatgggcgagagcctgaaccagccaagtcgcgtgaaggatgactgtcttatggattgtaaacttcttttatacgggaataacaagagccacgtgtggctccctgcatgtaccgtatgaataagcatcggctaactccgtgccagcagccgcggtaatacggaggatgcgagcgttatccggatttattgggtttaaagggtgcgtaggcggcctgttaagtaagtggttaaattgttgggctcaacccaatccagccacttaaactggcaggctagagtattggagaggcaagtggaattccatgtgtagcggtaaaatgcgtagatatatggaggaataccgatggcgaaggcagcctcctgggataacactgacgttcatgctcgaaagcgtgggtagcaaac

SEQ ID NO: 17 - DNA, 418 bp, Porphyromona
  misc_feature (1)..(418): Representative sequence
aggaatcttccacaatgggcgaaagcctgatggagcaacgccgcgtgaaggatgaaggccttcgggttgtaaacttcttttgtaggggaataaagaatggtacgtgtaccatagtgaatgtaccctacgaataagcatcggctaactccgtgccagcagccgcggtaatacggaggatgcgagcgttatccggatttattgggtttaaagggtgcgtaggcggcctgttaagtcagcggtgaaatctaggggcttaactcctaaattgccattgatactggtgggcttgagtgtagatgaggtaggcggaatgcgtggtgtagcggtggaatgcatagatatcacgcagaactccaattgcgaaggcagcttactaaggtacaactgacgctgaagcacgaaagcgtgggtatcaaac

SEQ ID NO: 18 - DNA, 399 bp, Porphyromona
  misc_feature (1)..(399): Representative sequence
gggaatattgcacaatgggggaaaccctgatgcagcgacgccgcgtgagtgaagaagtatttcggtatgtaaagctctatcagcagggaagataatgacagtacctgactaagaagccccggctaactacgtgccagcagccgcggtaatacggaggatgcgagcgttatccggatttattgggtttaaagggtgcgtaggcggcctgttaagtcagcggtgaaatctaggagcttaactcctaaattgccattgatactggcgggcttgagtgtagatgaggtaggcggaatgcgtggtgtagcggtggaatgcatagatatcacgcagaactccgattgcgaaggcagcttactaaggtacaactgacgctgaagcacgaaagcgtgggtatcaaac

SEQ ID NO: 19 - DNA, 401 bp, Fretibacterium
  misc_feature (1)..(401): Representative sequence
gggaatattgggcaatgggaggaatcctgacccagcgacgccgcgtgaacgaagacggccttcgggttgtaaagttcttttatgtgggaagaatgaagtgacggtaccacatgaataagccccggctaactacgtgccagcagccgcggtaatacgtagggggcgagcgttgtccggaattactgggcgtaaagggcacgcaggctgtgcttcaagtcagctgtaaaaggatgcggcttaaccgtgttatgcggctgagactgaggtgctggagtaccggagaggcaagtggaattcccagtgtagcggtgaaatgcgtagatattgggaagaacatcggtggcgaaggcgacttgctggacggtaactgacgctgaggtgcgaaagccagggtagcgaac

SEQ ID NO: 20 - DNA, 401 bp, Fretibacterium
  misc_feature (1)..(401): Representative sequence
gggaatattgggcaatgggaggaatcctgacccagcgacgccgcgtgaacgaagacggccttcgggttgtaaagttcttttatgtgggaagaaggaagtgacggtaccacatgaataagccccggctaactacgtgccagcagccgcggtaatacgtagggggcgagcgttgtccggaattactgggcgtaaagggcacgcaggctgtgcttcaagtcagctgtaaaaggatgcggcttaaccgtgttatgcggctgagactgaggtgctggagtaccggagaggcaagtggaattcccagtgtagcggtgaaatgcgtagatattgggaagaacatcggtggcgaaggcgacttgctggacggtaactgacgctgaggtgcgaaagccagggtagcgaac

SEQ ID NO: 21 - DNA, 401 bp, Fretibacterium
  misc_feature (1)..(401): Representative sequence
gggaatattgggcaatgggaggaatcctgacccagcgacgccgcgtgaacgaagacggccttcgggttgtaaagttcttttatgtgggaagaataaagtgacggtaccacatgaataagccccggctaactacgtgccagcagccgcggtaatacgtagggggcgagcgttgtccggaattactgggcgtaaagggcacgcaggctgtgcttcaagtcagctgtaaaaggatgcggcttaaccgtgttatgcagttgagactgaggtgctggagtaccggagaggcaagtggaattcccagtgtagcggtgaaatgcgtagatattgggaagaacatcggtggcgaaggcgacttgctggacggtaactgacgctgaggtgcgaaagccagggtagcgaac